European Patent Application EP 4 371 572 A1, published May 22, 2024. Title: ANTIBODY THAT SPECIFICALLY RECOGNIZES CD40 AND APPLICATION THEREOF. Applicant: STAIDSON (BEIJING) BIOPHARMACEUTICALS CO., LTD. The sequence listing filed with the application follows.

SEQUENCE LISTING (149 sequences)

SEQ ID NO: 1 - protein, 5 aa, Artificial Sequence
GYTVN

SEQ ID NO: 2 - protein, 5 aa, Artificial Sequence
GYVVN

SEQ ID NO: 3 - protein, 5 aa, Artificial Sequence
GYLVN

SEQ ID NO: 4 - protein, 5 aa, Artificial Sequence
DAYMH

SEQ ID NO: 5 - protein, 5 aa, Artificial Sequence
DSYMH

SEQ ID NO: 6 - protein, 5 aa, Artificial Sequence
DSYIH

SEQ ID NO: 7 - protein, 5 aa, Artificial Sequence
DHGMH

SEQ ID NO: 8 - protein, 5 aa, Artificial Sequence
DHAIH

SEQ ID NO: 9 - protein, 17 aa, Artificial Sequence
LINPYNGGTTYNQKFKG

SEQ ID NO: 10 - protein, 17 aa, Artificial Sequence
LINPRNGGTTYNQKFKG

SEQ ID NO: 11 - protein, 17 aa, Artificial Sequence
LINPYTGGTTYNQKFKG

SEQ ID NO: 12 - protein, 17 aa, Artificial Sequence
LINPKNGGTTYNQKFKG

SEQ ID NO: 13 - protein, 17 aa, Artificial Sequence
LINPYNGRTTYNQKFKG

SEQ ID NO: 14 - protein, 17 aa, Artificial Sequence
LIVPYNGGTTYNQKFKG

SEQ ID NO: 15 - protein, 17 aa, Artificial Sequence
LINPYSGGTTYNQKFKG

SEQ ID NO: 16 - protein, 17 aa, Artificial Sequence
LINPMNGGTTYNQKFKG

SEQ ID NO: 17 - protein, 17 aa, Artificial Sequence
LINPYNGGTWYNQKFKG

SEQ ID NO: 18 - protein, 17 aa, Artificial Sequence
LINPYNGGTSYNQKFKG

SEQ ID NO: 19 - protein, 17 aa, Artificial Sequence
LINPYHGGTTYNQKFKG

SEQ ID NO: 20 - protein, 17 aa, Artificial Sequence
LINPLNGGTTYNQKFKG

SEQ ID NO: 21 - protein, 17 aa, Artificial Sequence
LIAPYNGGTTYNQKFKG

SEQ ID NO: 22 - protein, 17 aa, Artificial Sequence
MINPYNGGTTYNQKFKG

SEQ ID NO: 23 - protein, 17 aa, Artificial Sequence
LINPTNGGTSYNQKFKG

SEQ ID NO: 24 - protein, 17 aa, Artificial Sequence
LINPSNGGTTYNQKFKG

SEQ ID NO: 25 - protein, 17 aa, Artificial Sequence
LINPYNGGTAYNQKFKG

SEQ ID NO: 26 - protein, 17 aa, Artificial Sequence
LINPENGGTTYNQKFKG

SEQ ID NO: 27 - protein, 17 aa, Artificial Sequence
RIDPANGNTKYDPKFQG

SEQ ID NO: 28 - protein, 17 aa, Artificial Sequence
RIDPTNGNTNFDPKFRG

SEQ ID NO: 29 - protein, 17 aa, Artificial Sequence
VISTSYGVATYNQKFKG

SEQ ID NO: 30 - protein, 17 aa, Artificial Sequence
AISTNYGAATYNQKFKG

SEQ ID NO: 31 - protein, 17 aa, Artificial Sequence
RIDPANGYTKSDPKFQG

SEQ ID NO: 32 - protein, 11 aa, Artificial Sequence
SYYSNPYAMDY

SEQ ID NO: 33 - protein, 11 aa, Artificial Sequence
SYYSKPYAMDY

SEQ ID NO: 34 - protein, 11 aa, Artificial Sequence
SYYSNPYANDY

SEQ ID NO: 35 - protein, 11 aa, Artificial Sequence
SLYSNPYAMDY

SEQ ID NO: 36 - protein, 11 aa, Artificial Sequence
SGYSNPYAMDY

SEQ ID NO: 37 - protein, 11 aa, Artificial Sequence
SYYSRPYAMDY

SEQ ID NO: 38 - protein, 11 aa, Artificial Sequence
SYYSNPYAGDY

SEQ ID NO: 39 - protein, 11 aa, Artificial Sequence
SMYSNPYAMDY

SEQ ID NO: 40 - protein, 11 aa, Artificial Sequence
SYYSNPYAADY

SEQ ID NO: 41 - protein, 11 aa, Artificial Sequence
SSYSNPYAMDY

SEQ ID NO: 42 - protein, 11 aa, Artificial Sequence
SYYSTPYAMDY

SEQ ID NO: 43 - protein, 11 aa, Artificial Sequence
SRYSNPYAMDY

SEQ ID NO: 44 - protein, 11 aa, Artificial Sequence
SYYSVPYAMDY

SEQ ID NO: 45 - protein, 11 aa, Artificial Sequence
SYYSNPYAQDY

SEQ ID NO: 46 - protein, 11 aa, Artificial Sequence
SYWSNPYAMDY

SEQ ID NO: 47 - protein, 11 aa, Artificial Sequence
SPYSNPYAMDY

SEQ ID NO: 48 - protein, 11 aa, Artificial Sequence
SYYSNPYASDY

SEQ ID NO: 49 - protein, 11 aa, Artificial Sequence
SYYSLPYAMDY

SEQ ID NO: 50 - protein, 11 aa, Artificial Sequence
SIYSNPYAMDY

SEQ ID NO: 51 - protein, 11 aa, Artificial Sequence
SYYVNPYAMDY

SEQ ID NO: 52 - protein, 11 aa, Artificial Sequence
SYYSDPYANDY

SEQ ID NO: 53 - protein, 11 aa, Artificial Sequence
NYYGSRYPFAY

SEQ ID NO: 54 - protein, 11 aa, Artificial Sequence
NYYGAAYPFAY

SEQ ID NO: 55 - protein, 11 aa, Artificial Sequence
NYYGSRYPFSY

SEQ ID NO: 56 - protein, 9 aa, Artificial Sequence
RDSKSPFDY

SEQ ID NO: 57 - protein, 10 aa, Artificial Sequence
RGSHGDWFAY

SEQ ID NO: 58 - protein, 11 aa, Artificial Sequence
KASQNVHTAVA

SEQ ID NO: 59 - protein, 11 aa, Artificial Sequence
KASQNVHTRVA

SEQ ID NO: 60 - protein, 11 aa, Artificial Sequence
KASQNVHTNVA

SEQ ID NO: 61 - protein, 11 aa, Artificial Sequence
KASQNVHTHVA

SEQ ID NO: 62 - protein, 10 aa, Artificial Sequence
SASSSVSYMH

SEQ ID NO: 63 - protein, 10 aa, Artificial Sequence
SGSSSVSYMH

SEQ ID NO: 64 - protein, 12 aa, Artificial Sequence
SASSSISSNYLH

SEQ ID NO: 65 - protein, 7 aa, Artificial Sequence
LASDRRT

SEQ ID NO: 66 - protein, 7 aa, Artificial Sequence
LRSDRRT

SEQ ID NO: 67 - protein, 7 aa, Artificial Sequence
STSNLAS

SEQ ID NO: 68 - protein, 7 aa, Artificial Sequence
FTSNLAS

SEQ ID NO: 69 - protein, 7 aa, Artificial Sequence
RTSNLAS

SEQ ID NO: 70 - protein, 9 aa, Artificial Sequence
LQHWNYPLT

SEQ ID NO: 71 - protein, 9 aa, Artificial Sequence
LQHWTYPLT

SEQ ID NO: 72 - protein, 9 aa, Artificial Sequence
LQAWNYPLT

SEQ ID NO: 73 - protein, 9 aa, Artificial Sequence
LQHWNSPLT

SEQ ID NO: 74 - protein, 9 aa, Artificial Sequence
LQHWNRPLT

SEQ ID NO: 75 - protein, 9 aa, Artificial Sequence
LQHWSYPLT

SEQ ID NO: 76 - protein, 9 aa, Artificial Sequence
LQHWNAPLT

SEQ ID NO: 77 - protein, 9 aa, Artificial Sequence
LQHWNQPLT

SEQ ID NO: 78 - protein, 9 aa, Artificial Sequence
QQGSSYPLT

SEQ ID NO: 79 - protein, 9 aa, Artificial Sequence
QQGSTYPLT

SEQ ID NO: 80 - protein, 9 aa, Artificial Sequence
HQYHRSPLT

SEQ ID NO: 81 - protein, 5 aa, Artificial Sequence
  VARIANT 3: note = X=L, T or V
GYXVN

SEQ ID NO: 82 - protein, 17 aa, Artificial Sequence
  VARIANT 1: note = X = L or M
  VARIANT 3: note = X = A, N, or V
  VARIANT 5: note = X = E, K, L, M, R, S, T, or Y
  VARIANT 6: note = X = H, N, S, or T
  VARIANT 8: note = X = G or R
  VARIANT 10: note = X = A, S, T, or W
XIXPXXGXTXYNQKFKG

SEQ ID NO: 83 - protein, 11 aa, Artificial Sequence
  VARIANT 2: note = X = G, I, L, M, P, R, S, or Y
  VARIANT 3: note = X = W or Y
  VARIANT 4: note = X = S or V
  VARIANT 5: note = X = D, K, L, N, R, T, or V
  VARIANT 9: note = X = A, G, M, N, Q, or S
SXXXXPYAXDY

SEQ ID NO: 84 - protein, 11 aa, Artificial Sequence
  VARIANT 9: note = X = A, H, N, or R
KASQNVHTXVA

SEQ ID NO: 85 - protein, 7 aa, Artificial Sequence
  VARIANT 2: note = X=A or R
LXSDRRT

SEQ ID NO: 86 - protein, 9 aa, Artificial Sequence
  VARIANT 3: note = X=A or H
  VARIANT 5: note = N, S or T
  VARIANT 6: note = X=A, Q, R, S or Y
LQXWXXPLT

SEQ ID NO: 87 - protein, 120 aa, Artificial Sequence
EVQLQQSGPDLVKPGASMKISCKASVYSFTGYTVNWVKQSHGKSLEWIGLINPYNGGTTYNQKFKGKATLTIDKSSTTAYMELLSLTSEDSAVYYCASSYYSNPYAMDYWGQGTSVTVSS

SEQ ID NO: 88 - protein, 120 aa, Artificial Sequence
QVQLVQSGAEVKKPGASVKVSCKASVYSFTGYTVNWVRQAPGQRLEWMGLINPYNGGTTYNQKFKGRVTLTIDKSASTAYMELSSLRSEDTAVYYCASSYYSNPYAMDYWGQGTLVTVSS

SEQ ID NO: 89 - protein, 120 aa, Artificial Sequence
QVQLVQSGAEVKKPGASVKVSCKASVYSFTGYTVNWVRQAPGQRLEWMGLINPRNGGTTYNQKFKGRVTLTIDKSASTAYMELSSLRSEDTAVYYCAWSYYSNPYAMDYWGQGTLVTVSS

SEQ ID NO: 90 - protein, 120 aa, Artificial Sequence
QVQLVQSGAEVKKPGASVKVSCKASVYSFTGYTVNWVRQAPGQRLEWMGLINPYTGGTTYNQKFKGRVTLTIDKSASTAYMELSSLRSEDTAVYYCASSYYSKPYAMDYWGQGTLVTVSS

SEQ ID NO: 91 - protein, 120 aa, Artificial Sequence
QVQLVQSGAEVKKPGASVKVSCKASVYGFTGYTVNWVRQAPGQRLEWMGLINPYNGGTTYNQKFKGRVTLTIDKSASTAYMELSSLRSEDTAVYYCASSYYSNPYANDYWGQGTLVTVSS

SEQ ID NO: 92 - protein, 120 aa, Artificial Sequence
QVQLVQSGAEVKKPGASVKVSCKASVYSFTGYTVNWVRQAPGQRLEWMGLINPKNGGTTYNQKFKGRVTLTIDKSASTAYMELSSLRSEDTAVYYCASSLYSNPYAMDYWGQGTLVTVSS

SEQ ID NO: 93 - protein, 120 aa, Artificial Sequence
QVQLVQSGAEVKKPGASVKVSCKASVYSFTGYVVNWVRQAPGQRLEWMGLINPYNGGTTYNQKFKGRVTLTIDKSASTAYMELSSLRSEDTAVYYCASSYYSNPYAMDYWGQGTLVTVSS

SEQ ID NO: 94 - protein, 120 aa, Artificial Sequence
QVQLVQSGAEVKKPGASVKVSCKASVYSFTGYTVNWVRQAPGQRLEWMGLINPYNGRTTYNQKFKGRVTLTIDKSASTAYMELSSLRSEDTAVYYCASSYYSNPYANDYWGQGTLVTVSS

SEQ ID NO: 95 - protein, 120 aa, Artificial Sequence
QVQLVQSGAEVKKPGASVKVSCKASVYSFTGYTVNWVRQAPGQRLEWMGLIVPYNGGTTYNQKFKGRVTLTIDKSASTAYMELSSLRSEDTAVYYCASSGYSNPYAMDYWGQGTLVTVSS

SEQ ID NO: 96 - protein, 120 aa, Artificial Sequence
QVQLVQSGAEVKKPGASVKVSCKASVYSFTGYTVNWVRQAPGQRLEWMGLINPYSGGTTYNQKFKGRVTLTIDKSASTAYMELSSLRSEDTAVYYCASSYYSRPYAMDYWGQGTLVTVSS

SEQ ID NO: 97 - protein, 120 aa, Artificial Sequence
QVQLVQSGAEVKKPGASVKVSCKASVYSFTGYTVNWVRQAPGQRLEWMGLINPMNGGTTYNQKFKGRVTLTIDKSASTAYMELSSLRSEDTAVYYCASSYYSNPYAGDYWGQGTLVTVSS

SEQ ID NO: 98 - protein, 120 aa, Artificial Sequence
QVQLVQSGAEVKKPGASVKVSCKASVYSFTGYTVNWVRQAPGQRLEWMGLINPYNGGTWYNQKFKGRVTLTIDKSASTAYMELSSLRSEDTAVYYCASSMYSNPYAMDYWGQGTLVTVSS

SEQ ID NO: 99 - protein, 120 aa, Artificial Sequence
QVQLVQSGAEVKKPGASVKVSCKASVYSFTGYTVNWVRQAPGQRLEWMGLINPYNGGTSYNQKFKGRVTLTIDKSASTAYMELSSLRSEDTAVYYCASSYYSNPYAADYWGQGTLVTVSS

SEQ ID NO: 100 - protein, 120 aa, Artificial Sequence
QVQLVQSGAEVKKPGASVKVSCKASVYSFTGYTVNWVRQAPGQRLEWMGLINPYHGGTTYNQKFKGRVTLTIDKSASTAYMELSSLRSEDTAVYYCASSSYSNPYAMDYWGQGTLVTVSS

SEQ ID NO: 101 - protein, 120 aa, Artificial Sequence
QVQLVQSGAEVKKPGASVKVSCKASVYSFTGYTVNWVRQAPGQRLEWMGLINPLNGGTTYNQKFKGRVTLTIDKSASTAYMELSSLRSEDTAVYYCASSYYSTPYAMDYWGQGTLVTVSS

SEQ ID NO: 102 - protein, 120 aa, Artificial Sequence
QVQLVQSGAEVKKPGASVKVSCKASVYSFTGYTVNWVRQAPGQRLEWMGLINPYNGGTTYNQKFKGRVTLTIDKSASTAYMELSSLRSEDTAVYYCASSYYSRPYAMDYWGQGTLVTVSS

SEQ ID NO: 103 - protein, 120 aa, Artificial Sequence
QVQLVQSGAEVKKPGASVKVSCKASVYSFTGYLVNWVRQAPGQRLEWMGLINPYNGGTTYNQKFKGRVTLTIDKSASTAYMELSSLRSEDTAVYYCASSYYSNPYAMDYWGQGTLVTVSS

SEQ ID NO: 104 - protein, 120 aa, Artificial Sequence
QVQLVQSGAEVKKPGASVKVSCKASVYSFTGYTVNWVRQAPGQRLEWMGLINPYNGGTTYNQKFKGRVTLTIDKSASTAYMELSSLRSEDTAVYYCASSRYSNPYAMDYWGQGTLVTVSS

SEQ ID NO: 105 - protein, 120 aa, Artificial Sequence
QVQLVQSGAEVKKPGASVKVSCKASVYSFTGYTVNWVRQAPGQRLEWMGLIAPYNGGTTYNQKFKGRVTLTIDKSASTAYMELSSLRSEDTAVYYCALSYYSNPYAMDYWGQGTLVTVSS

SEQ ID NO: 106 - protein, 120 aa, Artificial Sequence
QVQLVQSGAEVKKPGASVKVSCKASVYSFTGYTVNWVRQAPGQRLEWMGMINPYNGGTTYNQKFKGRVTLTIDKSASTAYMELSSLRSEDTAVYYCASSYYSVPYAMDYWGQGTLVTVSS

SEQ ID NO: 107 - protein, 120 aa, Artificial Sequence
QVQLVQSGAEVKKPGASVKVSCKASVYSFTGYTVNWVRQAPGQRLEWMGLINPYNGGTTYNQKFKGRVTLTIDKSASTAYMELSSLRSEDTAVYYCASSYYSNPYAQDYWGQGTLVTVSS

SEQ ID NO: 108 - protein, 120 aa, Artificial Sequence
QVQLVQSGAEVKKPGASVKVSCKASVYSFTGYTVNWVRQAPGQRLEWMGLINPYTGGTTYNQKFKGRVTLTIDKSASTAYMELSSLRSEDTAVYYCASSYWSNPYAMDYWGQGTLVTVSS

SEQ ID NO: 109 - protein, 120 aa, Artificial Sequence
QVQLVQSGAEVKKPGASVKVSCKASVYSFTGYTVNWVRQAPGQRLEWMGLINPYSGGTTYNQKFKGRVTLTIDKSASTAYMELSSLRSEDTAVYYCASSPYSNPYAMDYWGQGTLVTVSS

SEQ ID NO: 110 - protein, 120 aa, Artificial Sequence
QVQLVQSGAEVKKPGASVKVSCKASVYSFTGYTVNWVRQAPGQRLEWMGLIVPYNGGTTYNQKFKGRVTLTIDKSASTAYMELSSLRSEDTAVYYCASSRYSNPYAMDYWGQGTLVTVSS

SEQ ID NO: 111 - protein, 120 aa, Artificial Sequence
QVQLVQSGAEVKKPGASVKVSCKASVYSFTGYTVNWVRQAPGQRLEWMGLINPTNGGTSYNQKFKGRVTLTIDKSASTAYMELSSLRSEDTAVYYCASSYYSNPYASDYWGQGTLVTVSS

SEQ ID NO: 112 - protein, 120 aa, Artificial Sequence
QVQLVQSGAEVKKPGASVKVSCKASVYSFTGYTVNWVRQAPGQRLEWMGLINPYNGGTTYNQKFKGRVTLTIDKSASTAYMELSSLRSEDTAVYYCASSYYSLPYAMDYWGQGTLVTVSS

SEQ ID NO: 113 - protein, 120 aa, Artificial Sequence
QVQLVQSGAEVKKPGASVKVSCKASVYSFTGYTVNWVRQAPGQRLEWMGLINPYNGGTSYNQKFKGRVTLTIDKSASTAYMELSSLRSEDTAVYYCASSIYSNPYAMDYWGQGTLVTVSS

SEQ ID NO: 114 - protein, 120 aa, Artificial Sequence
QVQLVQSGAEVKKPGASVKVSCKASVYSFTGYTVNWVRQAPGQRLEWMGLINPYSGGTTYNQKFKGRVTLTIDKSASTAYMELSSLRSEDTAVYYCASSYYVNPYAMDYWGQGTLVTVSS

SEQ ID NO: 115 - protein, 120 aa, Artificial Sequence
QVQLVQSGAEVKKPGASVKVSCKASVYSFTGYTVNWVRQAPGQRLEWMGLINPYTGGTTYNQKFKGRVTLTIDKSASTAYMELSSLRSEDTAVYYCASSYYSNPYASDYWGQGTLVTVSS

SEQ ID NO: 116 - protein, 120 aa, Artificial Sequence
QVQLVQSGAEVKKPGASVKVSCKASVYSFTGYTVNWVRQAPGQRLEWMGLINPSNGGTTYNQKFKGRVTLTIDKSASTAYMELSSLRSEDTAVYYCASSYYSNPYANDYWGQGTLVTVSS

SEQ ID NO: 117 - protein, 120 aa, Artificial Sequence
QVQLVQSGAEVKKPGASVKVSCKASVYSFTGYTVNWVRQAPGQRLEWMGLINPYNGGTSYNQKFKGRVTLTIDKSASTAYMELSSLRSEDTAVYYCASSPYSNPYAMDYWGQGTLVTVSS

SEQ ID NO: 118 - protein, 120 aa, Artificial Sequence
QVQLVQSGAEVKKPGASVKVSCKASVYSFTGYTVNWVRQAPGQRLEWMGLINPYNGGTAYNQKFKGRVTLTIDKSASTAYMELSSLRSEDTAVYYCASSYYSDPYANDYWGQGTLVTVSS

SEQ ID NO: 119 - protein, 120 aa, Artificial Sequence
QVQLVQSGAEVKKPGASVKVSCKASVYSFTGYTVNWVRQAPGQRLEWMGLINPENGGTTYNQKFKGRVTLTIDKSASTAYMELSSLRSEDTAVYYCASSYYSNPYANDYWGQGTLVTVSS

SEQ ID NO: 120 - protein, 120 aa, Artificial Sequence
EVHVKQSGAELVKPGASVKLSCTASGFNIKDAYMHWVKQRPEQGLEWIGRIDPANGNTKYDPKFQGKASITTDTSSNTAYLQLSSLTSEDTAVYYCTPNYYGSRYPFAYWGQGTTVTVSS

SEQ ID NO: 121 - protein, 120 aa, Artificial Sequence
EVQLQQSGAELVKPGASVKLSCTASGFNIKDSYMHWVKQRPEQGLEWIGRIDPANGNTKYDPKFQGKATITADTSSNTAYLQLSSLTSEDTAVYYCVPNYYGAAYPFAYWGQGTTVTVSS

SEQ ID NO: 122 - protein, 120 aa, Artificial Sequence
EVMLVESGAELVRPGASVKLSCTASGFKIKDSYIHWMIQRPEQGLEWIGRIDPTNGNTNFDPKFRGKATLTTDTSSNTAYLQLSSLTSEDTAVYYCVPNYYGSRYPFSYWGQGTTVTVSS

SEQ ID NO: 123 - protein, 118 aa, Artificial Sequence
EVQLQQSGAELVSPGVSVKISCKGSGYTFTDHGMHWVKQSHAKSLEWIGVISTSYGVATYNQKFKGKATLSVDKSSSTAYLELARLTSEDSAIYYCARRDSKSPFDYWGQGTTLTVSS

SEQ ID NO: 124 - protein, 119 aa, Artificial Sequence
QVQLQQSGAELVRPGVSVKISCKGSGYTFTDHAIHWVKQSHARRLEWIGAISTNYGAATYNQKFKGKATMTVDKSSSTAYMELARLTSEDSAIYYCARRGSHGDWFAYWGQGTLVTVSA

SEQ ID NO: 125 - protein, 120 aa, Artificial Sequence
QIQLLQSGAELVKPGASVKLSCTASGFNIKDAYMHWVKQRPEQGLEWIGRIDPANGYTKSDPKFQGKATITSDTSSNTAYLQLSSLTSEDTAVYYCAPNYYGSRYPFAYWGQGTLVTVSS

SEQ ID NO: 126 - protein, 107 aa, Artificial Sequence
DIVLNQSQKFMSTSVGDRVSITCKASQNVHTAVAWYQQKPGQSPKALIYLASDRRTGIPDRFTGSGSGTDFTLTIDNVQSEDLADYFCLQHWNYPLTFGAGTKLELK

SEQ ID NO: 127 - protein, 107 aa, Artificial Sequence
EIVMTQSPATLSVSPGERATLSCKASQNVHTAVAWYQQKPGQAPRLLIYLASDRRTGIPARFSGSGSGTEFTLTISSLQSEDFAVYYCLQHWNYPLTFGQGTKVEIK

SEQ ID NO: 128 - protein, 107 aa, Artificial Sequence
EIVMTQSPATLSVSPGERATLSCKASQNVHTRVAWYQQKPGQAPRLLIYLASDRRTGIPARFSGSGSGTEFTLTISSLQSEDFAVYYCLQHWNYPLTFGQGTKVEIK

SEQ ID NO: 129 - protein, 107 aa, Artificial Sequence
EIVMTQSPATLSVSPGERATLSCKASQNVHTRVAWYQQKPGQAPRLLIYLASDRRTGIPARFSGSGSGTEFTLTISSLQSEDFAVYYCLQHWTYPLTFGQGTKVEIK

SEQ ID NO: 130 - protein, 107 aa, Artificial Sequence
EIVMTQSPATLSVSPGERATLSCKASQNVHTAVAWYQQKPGQAPRLLIYLRSDRRTGIPARFSGSGSGTEFTLTISSLQSEDFAVYYCLQAWNYPLTFGQGTKVEIK

SEQ ID NO: 131 - protein, 107 aa, Artificial Sequence
EIVMTQSPATLSVSPGERATLSCKASQNVHTNVAWYQQKPGQAPRLLIYLASDRRTGIPARFSGSGSGTEFTLTISSLQSEDFAVYYCLQHWNYPLTFGQGTKVEIK

SEQ ID NO: 132 - protein, 107 aa, Artificial Sequence
EIVMTQSPATLSVSPGERATLSCKASQNVHTRVAWYQQKPGQAPRLLIYLASDRRTGIPARFSGSGSGTEFTLTISSLQSEDFAVYYCLQHWNSPLTFGQGTKVEIK

SEQ ID NO: 133 - protein, 107 aa, Artificial Sequence
EIVMTQSPATLSVSPGERATLSCKASQNVHTRVAWYQQKPGQAPRLLIYLASDRRTGIPARFSGSGSGTEFTLTISSLQSEDFAVYYCLQHWNRPLTFGQGTKVEIK

SEQ ID NO: 134 - protein, 107 aa, Artificial Sequence
EIVMTQSPATLSVSPGERATLSCKASQNVHTRVAWYQQKPGQAPRLLIYLASDRRTGIPARFSGSGSGTEFTLTISSLQSEDFAVYYCLQHWSYPLTFGQGTKVEIK

SEQ ID NO: 135 - protein, 107 aa, Artificial Sequence
EIVMTQSPATLSVSPGERATLSCKASQNVHTHVAWYQQKPGQAPRLLIYLASDRRTGIPARFSGSGSGTEFTLTISSLQSEDFAVYYCLQHWNYPLTFGQGTKVEIK

SEQ ID NO: 136 - protein, 107 aa, Artificial Sequence
EIVMTQSPATLSVSPGERATLSCKASQNVHTRVAWYQQKPGQAPRLLIYLASDRRTGIPARFSGSGSGTEFTLTISSLQSEDFAVYYCLQHWNAPLTFGQGTKVEIK

SEQ ID NO: 137 - protein, 107 aa, Artificial Sequence
EIVMTQSPATLSVSPGERATMSCKASQNVHTRVAWYQQKPGQAPRLLIYLASDRRTGIPARFSGSGSGTEFTLTISSLQSEDFAVYYCLQHWNYPLTFGQGTKVEIK

SEQ ID NO: 138 - protein, 107 aa, Artificial Sequence
EIVMTQSPATLSVSPGERATLSCKASQNVHTRVAWYQQKPGQAPRLLIYLASDRRTGIPARFSGSGSGTEFTLTISSLQSEDFAVYYCLQHWNQPLTFGQGTKVEIK

SEQ ID NO: 139 - protein, 106 aa, Artificial Sequence
DIVLTQSPAIMSASPGEKVSITCSASSSVSYMHWFQQKPGTSPKLWIYSTSNLASGVPARFSGSGSGTSYSLTISRMEADDAATYYCQQGSSYPLTFGAGTKLELK

SEQ ID NO: 140 - protein, 106 aa, Artificial Sequence
DIVLIQSPAIMSASPGEKVTITCSASSSVSYMHWFQQKPGTSPKVWIYSTSNLASGVPARFGGSGSGTSYSLTISRMEAEDAATYYCQQGSSYPLTFGAGTKLELK

SEQ ID NO: 141 - protein, 106 aa, Artificial Sequence
QIVLTQSPAIMSASPGEKVTMTCSGSSSVSYMHWFQQKPGNSPKIWIYFTSNLASGVPARFSGSGSGTSYSLTISRMEAGDAATYYCQQGSTYPLTFGAGTKLELK

SEQ ID NO: 142 - protein, 108 aa, Artificial Sequence
QIVLTQSPAIMSASPGEKITITCSASSSISSNYLHWYQQKPGFSPKLLIYRTSNLASGVPARFSGSGSGTSYSLTISSMEAEDAATYYCHQYHRSPLTFGAGTKLELK

SEQ ID NO: 143 - protein, 106 aa, Artificial Sequence
DIELTQSPAIMSASPGEKVTITCSASSSVSYMHWFQQKPGTSPKLWIYSTSNLASGVPVRFSGSGSGTSYSLTISSMEAEDAATYYCHQYHRSPLTFGAGTKLELK

SEQ ID NO: 144 - protein, 106 aa, Artificial Sequence
QIVLTQSPAIMSASPGEKVTITCSASSSVSYMHWFQQKPGTSPKIWIYFTSNLASGVPARFSGSGSGTSYSLTISRMEAEDAATYYCQQGSTYPLTFGAGTKLELK

SEQ ID NO: 145 - protein, 330 aa, Artificial Sequence
ASTKGPSVFPLAPSSKSTSGGTAALGCLVKDYFPEPVTVSWNSGALTSGVHTFPAVLQSSGLYSLSSVVTVPSSSLGTQTYICNVNHKPSNTKVDKKVEPKSCDKTHTCPPCPAPELLGGPSVFLFPPKPKDTLMISRTPEVTCVVVDVSHEDPEVKFNWYVDGVEVHNAKTKPREEQYNSTYRVVSVLTVLHQDWLNGKEYKCKVSNKALPAPIEKTISKAKGQPREPQVYTLPPSREEMTKNQVSLTCLVKGFYPSDIAVEWESNGQPENNYKTTPPVLDSDGSFFLYSKLTVDKSRWQQGNVFSCSVMHEALHNHYTQKSLSLSPGK

SEQ ID NO: 146 - protein, 327 aa, Artificial Sequence
ASTKGPSVFPLAPCSRSTSESTAALGCLVKDYFPEPVTVSWNSGALTSGVHTFPAVLQSSGLYSLSSVVTVPSSSLGTKTYTCNVDHKPSNTKVDKRVESKYGPPCPSCPAPEFLGGPSVFLFPPKPKDTLMISRTPEVTCVVVDVSQEDPEVQFNWYVDGVEVHNAKTKPREEQFNSTYRVVSVLTVLHQDWLNGKEYKCKVSNKGLPSSIEKTISKAKGQPREPQVYTLPPSQEEMTKNQVSLTCLVKGFYPSDIAVEWESNGQPENNYKTTPPVLDSDGSFFLYSRLTVDKSRWQEGNVFSCSVMHEALHNHYTQKSLSLSLGK

SEQ ID NO: 147 - protein, 107 aa, Artificial Sequence [sequence omitted]

SEQ ID NO: 148 - protein, 106 aa, Artificial Sequence
GQPKAAPSVTLFPPSSEELQANKATLVCLISDFYPGAVTVAWKADSSPVKAGVETTTPSKQSNNKYAASSYLSLTPEQWKSHRSYSCQVTHEGSTVEKTVAPTECS

SEQ ID NO: 149 - protein, 277 aa, Artificial Sequence
MVRLPLQCVLWGCLLTAVHPEPPTACREKQYLINSQCCSLCQPGQKLVSDCTEFTETECLPCGESEFLDTWNRETHCHQHKYCDPNLGLRVQQKGTSETDTICTCEEGWHCTSEACESCVLHRSCSPGFGVKQIATGVSDTICEPCPVGFFSNVSSAFEKCHPWTSCETKDLVVQQAGTNKTDVVCGPQDRLRALVVIPIIFGILFAILLVLVFIKKVAKKPTNKAPHPKQEPQEINFPDDLPGSNTAAPVQETLHGCQPVTQEDGKESRISVQERQ